European Patent Application EP 4 293 360 A1, published December 20, 2023. Title: Methods and kits of testing adult onset still's disease and vasculitis. Applicant: CANON MEDICAL SYSTEMS CORPORATION General Incorporated Association The Japan-Multinational Trial Organization. The sequence listing filed with the application follows.

SEQUENCE LISTING (79 sequences)

SEQ ID NO: 1 - protein, 224 aa, Homo sapiens
MEKLLCFLVLTSLSHAFGQTDMSRKAFVFPKESDTSYVSLKAPLTKPLKAFTVCLHFYTELSSTRGYSIFSYATKRQDNEILIFWSKDIGYSFTVGGSEILFEVPEVTVAPVHICTSWESASGIVEFWVDGKPRVRKSLKKGYTVGAEASIILGQEQDSFGGNFEGSQSLVGDIGNVNMWDFVLSPDEINTIYLGGPFSPNVLNWRALKYEVQGEVFTKPQLWP

SEQ ID NO: 2 - protein, 10 aa, Artificial Sequence
  Epitope
EILFEVPEVT

SEQ ID NO: 3 - DNA, 1410 bp, Artificial Sequence
  Nucleotide sequence of polynucleotide encoding the heavy chain of the antibody 3C
atggaatggagctgggtctttctcttcctcctgtcagtaactgcaggtgtccaatcccaggttcagctgcagcagtctggggctgagctggtgaggcctggggcttcagtgaaactgtcctgcaaggctttggactacacatttactgactatgaaatgcactgggtgaaacagacacctgtgcatggcctggaatggattggagctattcatccaggaagaggtggtactgcctacaatcagaagttcaagggcaaggccacactgactgcagacaaatcctccagcacagcctacatggagctcagcagcctgacatctgaggactctggtgtctattactgtacaagttaccacggtggctactggggccaaggcaccactctcacagtctcctcagccaaaacaacacccccatcagtctatccactggcccctgggtgtggagatacaactggttcctccgtgactctgggatgcctggtcaagggctacttccctgagtcagtgactgtgacttggaactctggatccctgtccagcagtgtgcacaccttcccagctctcctgcagtctggactctacactatgagcagctcagtgactgtcccctccagcacctggccaagtcagaccgtcacctgcagcgttgctcacccagccagcagcaccacggtggacaaaaaacttgagcccagcgggcccatttcaacaatcaacccctgtcctccatgcaaggagtgtcacaaatgcccagctcctaacctcgagggtggaccatccgtcttcatcttccctccaaatatcaaggatgtactcatgatccccctgacacccaaggtcacgtgtgtggtggtggatgtgagcgaggatgacccagacgtccagatcagctggtttgtgaacaacgtggaagtacacacagctcagacacaaacccatagagaggattacaacagtactatccgggtggtcagcaccctccccatccagcaccaggactggatgagtggcaaggagttcaaatgcaaggtcaacaacaaagacctcccatcacccatcgagagaaccatctcaaaaattaaagggctagtcagagctccacaagtatacatcttgccgccaccagcagagcagttgtccaggaaagatgtcagtctcacttgcctggtcgtgggcttcaaccctggagacatcagtgtggagtggaccagcaatgggcatacagaggagaactacaaggacaccgcaccagtcctggactctgacggttcttacttcatatatagcaagctcaatatgaaaacaagcaagtgggagaaaacagattccttctcatgcaacgtgagacacgagggtctgaaaaattactacctgaagaagaccatctcccactctcctggtaaataa

SEQ ID NO: 4 - protein, 469 aa, Artificial Sequence
  Amino acid sequence of the heavy chain of the antibody 3C
MEWSWVFLFLLSVTAGVQSQVQLQQSGAELVRPGASVKLSCKALDYTFTDYEMHWVKQTPVHGLEWIGAIHPGRGGTAYNQKFKGKATLTADKSSSTAYMELSSLTSEDSGVYYCTSYHGGYWGQGTTLTVSSAKTTPPSVYPLAPGCGDTTGSSVTLGCLVKGYFPESVTVTWNSGSLSSSVHTFPALLQSGLYTMSSSVTVPSSTWPSQTVTCSVAHPASSTTVDKKLEPSGPISTINPCPPCKECHKCPAPNLEGGPSVFIFPPNIKDVLMIPLTPKVTCVVVDVSEDDPDVQISWFVNNVEVHTAQTQTHREDYNSTIRVVSTLPIQHQDWMSGKEFKCKVNNKDLPSPIERTISKIKGLVRAPQVYILPPPAEQLSRKDVSLTCLVVGFNPGDISVEWTSNGHTEENYKDTAPVLDSDGSYFIYSKLNMKTSKWEKTDSFSCNVRHEGLKNYYLKKTISHSPGK

SEQ ID NO: 5 - protein, 5 aa, Artificial Sequence
  CDR1 of Heavy chain found in the antibody 3C
DYEMH

SEQ ID NO: 6 - protein, 17 aa, Artificial Sequence
  CDR2 of Heavy chain found in the antibody 3C
AIHPGRGGTAYNQKFKG

SEQ ID NO: 7 - protein, 5 aa, Artificial Sequence
  CDR3 of Heavy chain found in the antibody 3C
YHGGY

SEQ ID NO: 8 - DNA, 717 bp, Artificial Sequence
  Nucleotide sequence of polynucleotide encoding the light chain of the antibody 3C
atgaagttgcctgttaggctgttggtgctgatgttctggattcctgctgcgagcagtgatgttgtgatgacccaaactccactctccctgcctgtcagtcttggagatcaagcctccatctcttgcagatctagtcagagccttgtacacagtaatgaaaacacctatttactttggtatctgcagaagccaggccagtctccaaagctcctgatctacaaagtttccaaccgattttctggggtcccagacaggttcagtggcagtggatcagggacagatttcacactcaagatcagcagagtggaggctgaggatctgggagtttatttctgctctcaaactacacatgttccgtggacgttcggtggaggcaccaagctggaaatcaaacgggctgatgctgcaccaactgtatccatcttcccaccatccagtgagcagttaacatctggaggtgcctcagtcgtgtgcttcttgaacaacttctaccccaaagacatcaatgtcaagtggaagattgatggcagtgaacgacaaaatggcgtcctgaacagttggactgatcaggacagcaaagacagcacctacagcatgagcagcaccctcacgttgaccaaggacgagtatgaacgacataacagctatacctgtgaggccactcacaagacatcaacttcacccattgtcaagagcttcaacaggaatgagtgttag

SEQ ID NO: 9 - protein, 238 aa, Artificial Sequence
  Amino acid sequence of the light chain of the antibody 3C
MKLPVRLLVLMFWIPAASSDVVMTQTPLSLPVSLGDQASISCRSSQSLVHSNENTYLLWYLQKPGQSPKLLIYKVSNRFSGVPDRFSGSGSGTDFTLKISRVEAEDLGVYFCSQTTHVPWTFGGGTKLEIKRADAAPTVSIFPPSSEQLTSGGASVVCFLNNFYPKDINVKWKIDGSERQNGVLNSWTDQDSKDSTYSMSSTLTLTKDEYERHNSYTCEATHKTSTSPIVKSFNRNEC

SEQ ID NO: 10 - protein, 16 aa, Artificial Sequence
  CDR1 of light chain found in the antibody 3C
RSSQSLVHSNENTYLL

SEQ ID NO: 11 - protein, 7 aa, Artificial Sequence
  CDR2 of light chain found in the antibody 3C
KVSNRFS

SEQ ID NO: 12 - protein, 9 aa, Artificial Sequence
  CDR3 of light chain found in the antibody 3C
SQTTHVPWT

SEQ ID NO: 13 - DNA, 1398 bp, Artificial Sequence
  Nucleotide sequence of polynucleotide encoding the heavy chain of the antibody 12C
atgaaatgcagctggatcatcttcttcctgatggcagtggttacaggggtcaattcagaggttcagctgcagcagtctggggcagagcttgtgaagccaggggcctcagtcaagttgtcctgcacagcttctggcttcaacattaaagactactatatacactgggtgaaacagaggactgatcagggcctggagtggattggaaggattgatcctgaagatgatgaaactaaatatgccccgaaattccagggcaaggccactataataacagacacatcctccaacacagcctacctgcacctcagcagcctgacatctgcggacactgccgtctattattgtgctagtcgaatttattattacgatattaagggcctttttgactactggggccaaggcaccactctcacagtctcctcagccaaaacgacacccccatctgtctatccactggcccctggatctgctgcccaaactaactccatggtgaccctgggatgcctggtcaagggctatttccctgagccagtgacagtgacctggaactctggatccctgtccagcggtgtgcacaccttcccagctgtcctgcagtctgacctctacactctgagcagctcagtgactgtcccctccagcacctggcccagccagaccgtcactgcaacgttgcccacccggccagcagcaccaaggtggacaagaaaattgtgcccagggattgtggttgtaagctttgcatatgtacagtcccagaagtatcatctgtcttcatcttcccccccaaagcccaaggatgtgctcaccattactctgactcctaaggtcacgtgtgttgtggtagacatcagcaaggatgatcccgaggtccagttcagctggtttgtagatgatgtggaggtgcacacagctcagacgaaaccccgggaggagcagatcaacagcactttccgttcagtcagtgaacttcccatcatgcaccaggactggctcaatggcaaggagttcaaatgcagggtcaacagtgcagctttccctgcccccatcgagaaaaccatctccaaaaccaaaggcagaccgaaggctccacaggtgtacaccattccacctcccaaggagcagatggccaaggataaagtcagtctgacctgcatgataacaaacttcttccctgaagacattactgtggagtggcagtggaatgggcagccagcggagaactacaagaacactcagcccatcatggacacagatggctcttacttcgtctacagcaagctcaatgtgcagaagagcaactgggaggcaggaaatactttcacctgctctgtgttacatgagggcctgcacaaccaccatactgagaagagcctctcccactctcctggtaaataa

SEQ ID NO: 14 - protein, 465 aa, Artificial Sequence
  Amino acid sequence of the heavy chain of the antibody 12C
MKCSWIIFFLMAVVTGVNSEVQLQQSGAELVKPGASVKLSCTASGFNIKDYYIHWVKQRTDQGLEWIGRIDPEDDETKYAPKFQGKATIITDTSSNTAYLHLSSLTSADTAVYYCASRIYYYDIKGLFDYWGQGTTLTVSSAKTTPPSVYPLAPGSAAQTNSMVTLGCLVKGYFPEPVTVTWNSGSLSSGVHTFPAVLQSDLYTLSSSVTVPSSTWPSQTVTATLPTRPAAPRWTRKLCPGIVVVSFAYVQSQKYHLSSSSPPKPKDVLTITLTPKVTCVVVDISKDDPEVQFSWFVDDVEVHTAQTKPREEQINSTFRSVSELPIMHQDWLNGKEFKCRVNSAAFPAPIEKTISKTKGRPKAPQVYTIPPPKEQMAKDKVSLTCMITNFFPEDITVEWQWNGQPAENYKNTQPIMDTDGSYFVYSKLNVQKSNWEAGNTFTCSVLHEGLHNHHTEKSLSHSPGK

SEQ ID NO: 15 - protein, 5 aa, Artificial Sequence
  CDR1 of heavy chain found in the antibody 12C
DYYIH

SEQ ID NO: 16 - protein, 17 aa, Artificial Sequence
  CDR2 of heavy chain found in the antibody 12C
RIDPEDDETKYAPKFQG

SEQ ID NO: 17 - protein, 13 aa, Artificial Sequence
  CDR3 of heavy chain found in the antibody 12C
RIYYYDIKGLFDY

SEQ ID NO: 18 - DNA, 723 bp, Artificial Sequence
  Nucleotide sequence of polynucleotide encoding the light chain of the antibody 12C
atggaatcacagactcaggtcctcatgtccctgctgttctgggtatctggtacctgtggggacattgtgatgacacaggctccatcctccctgactgtgacagcaggagagaaggtcactatgacctgcaagtccagtcagagtctgttaaatagtggaaatcaaaagaactacttgacctggtcccagcagaaaccagggcagcctcctaaactgttgatctactgggcatccactagggaatctggggtccctgatcgcttcacaggcagtggatctggaacagatttcactctcaccatcagcagtgtgcaggctgaagacctggcagtttattactgtcagaatgattataattatccgatcacgttcggtgctgggaccaagctggagctgaaacgggctgatgctgcaccaactgtatccatcttcccaccatccagtgagcagttaacatctggaggtgcctcagtcgtgtgcttcttgaacaacttctaccccaaagacatcaatgtcaagtggaagattgatggcagtgaacgacaaaatggcgtcctgaacagttggactgatcaggacagcaaagacagcacctacagcatgagcagcaccctcacgttgaccaaggacgagtatgaacgacataacagctatacctgtgaggccactcacaagacatcaacttcacccattgtcaagagcttcaacaggaatgagtgttag

SEQ ID NO: 19 - protein, 240 aa, Artificial Sequence
  Amino acid sequence of the light chain of the antibody 12C
MESQTQVLMSLLFWVSGTCGDIVMTQAPSSLTVTAGEKVTMTCKSSQSLLNSGNQKNYLTWSQQKPGQPPKLLIYWASTRESGVPDRFTGSGSGTDFTLTISSVQAEDLAVYYCQNDYNYPITFGAGTKLELKRADAAPTVSIFPPSSEQLTSGGASVVCFLNNFYPKDINVKWKIDGSERQNGVLNSWTDQDSKDSTYSMSSTLTLTKDEYERHNSYTCEATHKTSTSPIVKSFNRNEC

SEQ ID NO: 20 - protein, 17 aa, Artificial Sequence
  CDR1 of light chain found in the antibody 12C
KSSQSLLNSGNQKNYLT

SEQ ID NO: 21 - protein, 7 aa, Artificial Sequence
  CDR2 of light chain found in the antibody 12C
WASTRES

SEQ ID NO: 22 - protein, 9 aa, Artificial Sequence
  CDR3 of light chain found in the antibody 12C
QNDYNYPIT

SEQ ID NO: 23 - DNA, 1431 bp, Artificial Sequence
  Nucleotide sequence of polynucleotide encoding the heavy chain of the antibody 18A
atgaaatgcagctggatcatcttcttcctgatggcagtggttacaggggtcaattcagaggttcagctgcagcagtctggggcagagtttgtgaagccagggacctcagtcaagttgtcctgcacagcttctggcttcaacattaaagactactatattcactgggtgaagcagaggactgaacagggcctggagtggattggaaggattgatcctgaggatggtgaaactaaatatgccccgaaattccagggcaaggccactataacagcagacgcttcctccaacacagcctacctgcagctcagcagcctgacatctgaggacactgccgtctattactgtgttagtcgaatgtattactacggtagtcagggcctttttgacttctggggccaaggcaccactctcacagtctcctcagccaaaacaacagccccatcggtctatccactggcccctgtgtgtggaggtacaactggctcctcggtgactctaggatgcctggtcaagggttatttccctgagccagtgaccttgacctggaactctggatccctgtccagtggtgtgcacaccttcccagctctcctgcagtctggcctctacaccctcagcagctcagtgactgtaacctcgaacacctggcccagccagaccatcacctgcaatgtggcccacccggcaagcagcaccaaagtggacaagaaaattgagcccagagtgcccataacacagaacccctgtcctccactcaaagagtgtcccccatgcgcagctccagacctcttgggtggaccatccgtcttcatcttccctccaaagatcaaggatgtactcatgatctccctgagccccatggtcacatgtgtggtggtggatgtgagcgaggatgacccagacgtccagatcagctggtttgtgaacaacgtggaagtacacacagctcagacacaaacccatagagaggattacaacagtactctccgggtggtcagtgccctccccatccagcaccaggactggatgagtggcaaggagttcaaatgcaaggtcaacaacagagccctcccatcccccatcgagaaaaccatctcaaaacccagagggccagtaagagctccacaggtatatgtcttgcctccaccagcagaagagatgactaagaaagagttcagtctgacctgcatgatcacaggcttcttacctgccgaaattgctgtggactggaccagcaatgggcgtacagagcaaaactacaagaacaccgcaacagtcctggactctgatggttcttacttcatgtacagcaagctcagagtacaaaagagcacttgggaaagaggaagtcttttcgcctgctcagtggtccacgagggtctgcacaatcaccttacgactaagaccatctcccactctcctggtaaataa

SEQ ID NO: 24 - protein, 476 aa, Artificial Sequence
  Amino acid sequence of the heavy chain of the antibody 18A
MKCSWIIFFLMAVVTGVNSEVQLQQSGAEFVKPGTSVKLSCTASGFNIKDYYIHWVKQRTEQGLEWIGRIDPEDGETKYAPKFQGKATITADASSNTAYLQLSSLTSEDTAVYYCVSRMYYYGSQGLFDFWGQGTTLTVSSAKTTAPSVYPLAPVCGGTTGSSVTLGCLVKGYFPEPVTLTWNSGSLSSGVHTFPALLQSGLYTLSSSVTVTSNTWPSQTITCNVAHPASSTKVDKKIEPRVPITQNPCPPLKECPPCAAPDLLGGPSVFIFPPKIKDVLMISLSPMVTCVVVDVSEDDPDVQISWFVNNVEVHTAQTQTHREDYNSTLRVVSALPIQHQDWMSGKEFKCKVNNRALPSPIEKTISKPRGPVRAPQVYVLPPPAEEMTKKEFSLTCMITGFLPAEIAVDWTSNGRTEQNYKNTATVLDSDGSYFMYSKLRVQKSTWERGSLFACSVVHEGLHNHLTTKTISHSPGK

SEQ ID NO: 25 - protein, 5 aa, Artificial Sequence
  CDR1 of heavy chain found in the antibody 18A
DYYIH

SEQ ID NO: 26 - protein, 17 aa, Artificial Sequence
  CDR2 of heavy chain found in the antibody 18A
RIDPEDGETKYAPKFQG

SEQ ID NO: 27 - protein, 13 aa, Artificial Sequence
  CDR3 of heavy chain found in the antibody 18A
RMYYYGSQGLFDF

SEQ ID NO: 28 - DNA, 723 bp, Artificial Sequence
  Nucleotide sequence of polynucleotide encoding the light chain of the antibody 18A
atggaatcacagactcaggtcctcatgtccctgctgttctgggtatctggtacctgtggggacattgtgatgacacagtctccatcctccctgactgtgacagcaggagagaaggtcactatgggctgtaagtccagtcagagtctgttaaacagtgcaaatcaaaagaactacttgacctggtaccggcagaaaccagggcagcctcctaaactgttgatctactgggcttccactagggaatctggggtccctgatcgcttcacaggcagtggatctggaacagatttcactctcaccatcagcagtgtgcaggctgaagacctggcagtttattactgtcagaatgattataattatccgctcacgtgcggtgctgggaccaagctggacctgaaacgggctgatgctgcaccaactgtatccatcttcccaccatccagtgagcagttaacatctggaggtgcctcagtcgtgtgcttcttgaacaacttctaccccaaagacatcaatgtcaagtggaagattgatggcagtgaacgacaaaatggcgtcctgaacagttggactgatcaggacagcaaagacagcacctacagcatgagcagcaccctcacgttgaccaaggacgagtatgaacgacataacagctatacctgtgaggccactcacaagacatcaacttcacccattgtcaagagcttcaacaggaatgagtgttag

SEQ ID NO: 29 - protein, 240 aa, Artificial Sequence
  Amino acid sequence of the light chain of the antibody 18A
MESQTQVLMSLLFWVSGTCGDIVMTQSPSSLTVTAGEKVTMGCKSSQSLLNSANQKNYLTWYRQKPGQPPKLLIYWASTRESGVPDRFTGSGSGTDFTLTISSVQAEDLAVYYCQNDYNYPLTCGAGTKLDLKRADAAPTVSIFPPSSEQLTSGGASVVCFLNNFYPKDINVKWKIDGSERQNGVLNSWTDQDSKDSTYSMSSTLTLTKDEYERHNSYTCEATHKTSTSPIVKSFNRNEC

SEQ ID NO: 30 - protein, 17 aa, Artificial Sequence
  CDR1 of light chain found in the antibody 18A
KSSQSLLNSANQKNYLT

SEQ ID NO: 31 - protein, 7 aa, Artificial Sequence
  CDR2 of light chain found in the antibody 18A
WASTRES

SEQ ID NO: 32 - protein, 9 aa, Artificial Sequence
  CDR3 of light chain found in the antibody 18A
QNDYNYPLT

SEQ ID NO: 33 - protein, 11 aa, Artificial Sequence
  Partial peptide of human CRP
QTDMSRKAFVC

SEQ ID NO: 34 - protein, 11 aa, Artificial Sequence
  Partial peptide of human CR
FPKESDTSYVC

SEQ ID NO: 35 - protein, 11 aa, Artificial Sequence
  Partial peptide of human CRP
SLKAPLTKPLC

SEQ ID NO: 36 - protein, 11 aa, Artificial Sequence
  Partial peptide of human CRP
KAFTVCLHFYC

SEQ ID NO: 37 - protein, 11 aa, Artificial Sequence
  Partial peptide of human CRP
TELSSTRGYSC

SEQ ID NO: 38 - protein, 11 aa, Artificial Sequence
  Partial peptide of human CRP
IFSYATKRQDC

SEQ ID NO: 39 - protein, 11 aa, Artificial Sequence
  Partial peptide of human CRP
NEILIFWSKDC

SEQ ID NO: 40 - protein, 11 aa, Artificial Sequence
  Partial peptide of human CRP
IGYSFTVGGSC

SEQ ID NO: 41 - protein, 11 aa, Artificial Sequence
  Partial peptide of human CRP
EILFEVPEVTC

SEQ ID NO: 42 - protein, 11 aa, Artificial Sequence
  Partial peptide of human CRP
VAPVHICTSWC

SEQ ID NO: 43 - protein, 11 aa, Artificial Sequence
  Partial peptide of human CRP
ESASGIVEFWC

SEQ ID NO: 44 - protein, 11 aa, Artificial Sequence
  Partial peptide of human CRP
VDGKPRVRKSC

SEQ ID NO: 45 - protein, 11 aa, Artificial Sequence
  Partial peptide of human CRP
LKKGYTVGAEC

SEQ ID NO: 46 - protein, 11 aa, Artificial Sequence
  Partial peptide of human CRP
ASIILGQEQDC

SEQ ID NO: 47 - protein, 11 aa, Artificial Sequence
  Partial peptide of human CRP
SFGGNFEGSQC

SEQ ID NO: 48 - protein, 11 aa, Artificial Sequence
  Partial peptide of human CRP
SLVGDIGNVNC

SEQ ID NO: 49 - protein, 11 aa, Artificial Sequence
  Partial peptide of human CRP
MWDFVLSPDEC

SEQ ID NO: 50 - protein, 11 aa, Artificial Sequence
  Partial peptide of human CRP
INTIYLGGPFC

SEQ ID NO: 51 - protein, 11 aa, Artificial Sequence
  Partial peptide of human CRP
SPNVLNWRALC

SEQ ID NO: 52 - protein, 17 aa, Artificial Sequence
  Partial peptide of human CRP
KYEVQGEVFTKPQLWPC

SEQ ID NO: 53 - protein, 31 aa, Artificial Sequence
  Partial peptide of human CRP
QTDMSRKAFVFPKESDTSYVSLKAPLTKPLC

SEQ ID NO: 54 - protein, 31 aa, Artificial Sequence
  Partial peptide of human CRP
KAFTVCLHFYTELSSTRGYSIFSYATKRQDC

SEQ ID NO: 55 - protein, 31 aa, Artificial Sequence
  Partial peptide of human CRP
NEILIFWSKDIGYSFTVGGSEILFEVPEVTC

SEQ ID NO: 56 - protein, 31 aa, Artificial Sequence
  Partial peptide of human CRP
VAPVHICTSWESASGIVEFWVDGKPRVRKSC

SEQ ID NO: 57 - protein, 31 aa, Artificial Sequence
  Partial peptide of human CRP
LKKGYTVGAEASIILGQEQDSFGGNFEGSQC

SEQ ID NO: 58 - protein, 31 aa, Artificial Sequence
  Partial peptide of human CRP
SLVGDIGNVNMWDFVLSPDEINTIYLGGPFC

SEQ ID NO: 59 - protein, 27 aa, Artificial Sequence
  Partial peptide of human CRP
SPNVLNWRALKYEVQGEVFTKPQLWPC

SEQ ID NO: 60 - DNA, 1389 bp, Artificial Sequence
  Heavy chain of chimeric antibody
atgggctggacattggtctttctcttcctgttgagcgtcactgcaggggtccactcacaggtgcaactgcagcagagtggggccgaactggttagacccggcgcaagtgttaagctgtcttgcaaggctctggactacaccttcactgactatgagatgcattgggtgaaacagacacctgtgcatggtctggaatggatcggagcaatacacccaggtcgaggaggaaccgcctataaccagaagtttaagggaaaagccaccttgactgctgataagtcctcttcaacagcctatatggagctttccagccttacttccgaggacagtggggtttactattgtaccagttatcacggaggttactggggacaggggaccacactgacagttagcagtgcctctacgaaaggcccctccgtgtttcctttggctccatcttcaaagtccacctcaggcggcaccgctgccctcggatgtctggtgaaggactacttccctgagcccgttactgtgtcatggaatagcggggctctgacttccggggtccacacatttcccgctgtacttcagtccagtggcttgtacagcctgtcctctgtggtcaccgttccaagctctagcctgggtacacagacctatatctgcaacgtaaaccataaaccctctaacacgaaggtagacaagaaagtcgagcctaagtcctgcgataagacccacacctgtccaccctgtcccgcacccgagctcctgggtggccctagcgtattcctgtttccacccaaaccaaaagacacactgatgatttccaggacacccgaggtgacatgcgtggtcgtggacgtgtctcatgaggaccccgaagtgaagttcaactggtatgttgatggagtcgaagtgcacaatgccaaaacgaagccacgcgaagaacagtacaactccacatatcgggtcgtatccgtcctgactgtgctccatcaggattggctgaatggcaaggagtacaaatgcaaggtgtccaataaggccttgcctgcacccatcgagaaaactatctccaaagccaaaggccagcctcgtgaacctcaagtgtacaccctgcctccatctagggatgagctgaccaagaaccaggtgtcactgacttgccttgtgaaaggcttttaccctagcgatattgctgttgaatgggagtccaatggtcagccagagaacaattacaagacaacccctccagtcctggactctgatgggagcttctttctctactctaagctcaccgtggataagagccggtggcaacaaggcaatgtgttcagttgttctgtgatgcatgaagccctccacaaccactatactcagaagtcactgagtcttagccccggtaaa

SEQ ID NO: 61 - protein, 463 aa, Artificial Sequence
  Heavy chain of chimeric antibody
MGWTLVFLFLLSVTAGVHSQVQLQQSGAELVRPGASVKLSCKALDYTFTDYEMHWVKQTPVHGLEWIGAIHPGRGGTAYNQKFKGKATLTADKSSSTAYMELSSLTSEDSGVYYCTSYHGGYWGQGTTLTVSSASTKGPSVFPLAPSSKSTSGGTAALGCLVKDYFPEPVTVSWNSGALTSGVHTFPAVLQSSGLYSLSSVVTVPSSSLGTQTYICNVNHKPSNTKVDKKVEPKSCDKTHTCPPCPAPELLGGPSVFLFPPKPKDTLMISRTPEVTCVVVDVSHEDPEVKFNWYVDGVEVHNAKTKPREEQYNSTYRVVSVLTVLHQDWLNGKEYKCKVSNKALPAPIEKTISKAKGQPREPQVYTLPPSRDELTKNQVSLTCLVKGFYPSDIAVEWESNGQPENNYKTTPPVLDSDGSFFLYSKLTVDKSRWQQGNVFSCSVMHEALHNHYTQKSLSLSPGK

SEQ ID NO: 62 - DNA, 1389 bp, Artificial Sequence
  Heavy chain of humanized antibody
atgggctggacgctcgtattcctctttcttctgtccgttacggcaggagtccactctcaggtgcagctggtccaatctggagctgaggtcaagaaaccaggcgctagcgtgatgttgagctgtaaagcctccgactacacatttaccgactacgagatgcactgggtgaaacaggctcctgtgcatggcctcgaatggattggcgcaatccatcccggaagaggaggtacagcctataaccagaagttcaaaggtcgggtgtccatgactcgagacacatctactagcacggtttatctggaactgagttctctgcgctctgaggatacagccgtgtattactgcaccagttaccatggcggctattggggtcaagggactttggtgacagtaagttccgcatccacaaagggtccatcagtctttccccttgcaccttcatccaagtccacatctggcgggacagctgccttggggtgcttggtcaaggactactttccagaaccagtgactgtcagttggaactctggagccctgacttctggagtgcataccttcccagccgtgctgcaatcaagcgggctgtacagtctgtccagtgtcgtgactgttccctcttcatccctcggtacccagacttacatctgcaatgtcaaccacaaacctagcaataccaaggtagacaagaaggtggagcccaaatcctgcgataagactcatacctgtcctccctgtcctgctcctgaacttcttggcggacccagtgtattcctgtttcctccaaagcccaaggacaccctcatgatcagcaggaccccagaagtgacctgtgtggtagtggacgtcagccacgaagatcccgaagtgaagttcaattggtacgttgatggcgtcgaggttcacaacgccaagaccaagcccagggaggaacagtacaattccacttatcgggttgtgtcagtgctgaccgttctgcatcaggattggcttaatggcaaggagtataagtgcaaggtttccaacaaagcactgccagctcctatcgagaaaaccattagcaaagccaaaggtcagccaagagagcctcaggtctatactctgcctccttctcgtgatgagctgaccaagaaccaggtcagcctgacatgtctcgtgaaagggttttaccccagcgacatagctgtggagtgggagtccaatgggcagcccgagaacaactacaagaccacaccacccgtgttggatagcgatggctccttctttctgtatagcaagctgacagttgacaagagtcgctggcaacaggggaatgtgttctcttgctcagtaatgcacgaagccctgcacaaccactatacccagaaatctctctccctgtcacccggaaaa

SEQ ID NO: 63 - protein, 463 aa, Artificial Sequence
  Heavy chain of humanized antibody
MGWTLVFLFLLSVTAGVHSQVQLVQSGAEVKKPGASVMLSCKASDYTFTDYEMHWVKQAPVHGLEWIGAIHPGRGGTAYNQKFKGRVSMTRDTSTSTVYLELSSLRSEDTAVYYCTSYHGGYWGQGTLVTVSSASTKGPSVFPLAPSSKSTSGGTAALGCLVKDYFPEPVTVSWNSGALTSGVHTFPAVLQSSGLYSLSSVVTVPSSSLGTQTYICNVNHKPSNTKVDKKVEPKSCDKTHTCPPCPAPELLGGPSVFLFPPKPKDTLMISRTPEVTCVVVDVSHEDPEVKFNWYVDGVEVHNAKTKPREEQYNSTYRVVSVLTVLHQDWLNGKEYKCKVSNKALPAPIEKTISKAKGQPREPQVYTLPPSRDELTKNQVSLTCLVKGFYPSDIAVEWESNGQPENNYKTTPPVLDSDGSFFLYSKLTVDKSRWQQGNVFSCSVMHEALHNHYTQKSLSLSPGK

SEQ ID NO: 64 - DNA, 1389 bp, Artificial Sequence
  Heavy chain of humanized antibody
atggggtggacacttgtctttctctttctgctgtctgttaccgctggcgtacactcccaagtacagctggtccaaagcggcgctgaagtcgtgcgacccggggcaagcgtgaaactgtcctgtaaagcctccgactatactttcactgattacgagatgcattgggtacgacaggcaccaggccagggtcttgagtgggttggcgctattcatcctggtcggggtggaaccgcctacaatcagaagttcaaaggccgcgtgacaattactgccgataagtcaacaagtaccgcttacatggaattgtcatccctgcgcagtgaggatactgccgtctactattgcacctcctatcatggaggatattggggccaagggactaccgtgaccgtaagttctgcctcaacaaaagggccctctgtgtttcccctggcaccctctagcaagagtacaagcggaggcacagctgccctgggttgtctggtgaaagactactttcctgagccagtcacagtgtcatggaatagcggagcactgacttctggagtgcacacctttcccgcagtcttgcagagttctggcctgtattccctctcctccgttgttacagtcccatcctcttctctcgggacccagacatacatctgcaacgtgaaccacaagcctagcaacacgaaggtggacaagaaagttgagcccaagagctgtgataagacccacacttgcccaccttgtccagcccctgaactccttggtggtccaagcgtgttcctctttccaccaaagcctaaggacaccttgatgatcagcaggactcctgaagtgacgtgtgtggtggtggacgtgtcccatgaagatcccgaggtcaagttcaattggtatgtagacggggtagaggttcacaacgctaaaacaaaaccccgtgaggagcagtacaacagcacatatcgggtcgtcagtgtccttaccgtgctgcatcaggattggctgaatggaaaggagtataagtgcaaagtgtccaacaaggccctgcccgctcccatcgagaaaaccatctctaaggctaaaggccagcccagagaacctcaggtgtataccctcccaccttcaagggacgaattgaccaagaatcaggtgtcccttacttgcttggttaaaggcttctacccctcagacatagccgttgagtgggaatcaaatggacagcctgagaacaactacaaaaccacgcctccagtgctggattccgatggctccttctttctgtactctaagctgacagtcgacaagagtagatggcagcaagggaatgtgttcagctgcagtgttatgcatgaagccctgcacaaccactacactcagaagtctctgagcctgtctcccggtaag

SEQ ID NO: 65 - protein, 463 aa, Artificial Sequence
  Heavy chain of humanized antibody
MGWTLVFLFLLSVTAGVHSQVQLVQSGAEVVRPGASVKLSCKASDYTFTDYEMHWVRQAPGQGLEWVGAIHPGRGGTAYNQKFKGRVTITADKSTSTAYMELSSLRSEDTAVYYCTSYHGGYWGQGTTVTVSSASTKGPSVFPLAPSSKSTSGGTAALGCLVKDYFPEPVTVSWNSGALTSGVHTFPAVLQSSGLYSLSSVVTVPSSSLGTQTYICNVNHKPSNTKVDKKVEPKSCDKTHTCPPCPAPELLGGPSVFLFPPKPKDTLMISRTPEVTCVVVDVSHEDPEVKFNWYVDGVEVHNAKTKPREEQYNSTYRVVSVLTVLHQDWLNGKEYKCKVSNKALPAPIEKTISKAKGQPREPQVYTLPPSRDELTKNQVSLTCLVKGFYPSDIAVEWESNGQPENNYKTTPPVLDSDGSFFLYSKLTVDKSRWQQGNVFSCSVMHEALHNHYTQKSLSLSPGK

SEQ ID NO: 66 - DNA, 1389 bp, Artificial Sequence
  Heavy chian of humanized antibody
atgggctggacactggtgtttctctttctccttagcgttaccgccggtgtgcactctcaggttcagctggtgcagtcaggagctgaggtgaagaaaccaggcgcttctgtgaaggtgtcttgtaaagcctctgactacactttcaccgactatgagatgcattgggtccggcagacacccggacatggccttgaatggatgggagccattcatcctggcagaggagggacagcctataaccagaagttcaagggacgcgttactatgaccgctgacaagtccatttccaccgcctacatggagctcaactcactgacttctgacgattcagccgtgtactactgtaccagctatcacggcgggtattggggacaggggaccctggtgactgtgtctagtgcaagcacaaaaggaccctctgttttccctctggctccttcctctaagagcacttcaggtggcaccgcagccttgggttgtctggtgaaggactactttccagaacctgtgacagtctcatggaactctggtgctctgacaagcggcgtgcatacttttccagctgtcctgcagagttccggcctgtattctctgtcctcagtcgtcactgtgccctctagttccttggggacccaaacctacatctgcaatgtcaatcacaaacctagtaatacgaaagtagacaagaaagtagagcccaagagctgcgacaagacccacacatgccctccatgtccagcacctgaattgctgggtggcccatccgtgtttctgtttcctcccaaaccaaaagatacactgatgatcagccggactcccgaagtgacctgtgtagttgtggacgtcagccatgaagatcccgaggtcaaattcaactggtatgttgatggtgtagaggttcacaatgccaagactaagccacgagaggaacagtacaatagcacctatcgtgtcgtaagtgtccttaccgtcctccaccaagactggcttaacggcaaagagtacaagtgcaaagtctctaacaaggcactccctgcaccaatcgagaaaacgatcagcaaggccaaggggcaacccagagaaccccaggtttatactctgccaccctccagggatgagttgacgaagaatcaggtgtccctgacatgcctcgtgaaagggttctaccccagtgatatagccgtagaatgggagtccaatggtcagcccgagaacaactacaagacaacacctcccgtgctggatagcgacggaagtttcttcctgtactccaagttgaccgtggataagtccaggtggcaacaggggaatgtgtttagctgctcagtgatgcacgaagctcttcacaaccattatacccagaaatccctgtccctgagtcctggcaag

SEQ ID NO: 67 - protein, 463 aa, Artificial Sequence
  Heavy chain of humanized antibody
MGWTLVFLFLLSVTAGVHSQVQLVQSGAEVKKPGASVKVSCKASDYTFTDYEMHWVRQTPGHGLEWMGAIHPGRGGTAYNQKFKGRVTMTADKSISTAYMELNSLTSDDSAVYYCTSYHGGYWGQGTLVTVSSASTKGPSVFPLAPSSKSTSGGTAALGCLVKDYFPEPVTVSWNSGALTSGVHTFPAVLQSSGLYSLSSVVTVPSSSLGTQTYICNVNHKPSNTKVDKKVEPKSCDKTHTCPPCPAPELLGGPSVFLFPPKPKDTLMISRTPEVTCVVVDVSHEDPEVKFNWYVDGVEVHNAKTKPREEQYNSTYRVVSVLTVLHQDWLNGKEYKCKVSNKALPAPIEKTISKAKGQPREPQVYTLPPSRDELTKNQVSLTCLVKGFYPSDIAVEWESNGQPENNYKTTPPVLDSDGSFFLYSKLTVDKSRWQQGNVFSCSVMHEALHNHYTQKSLSLSPGK

SEQ ID NO: 68 - DNA, 1389 bp, Artificial Sequence
  Heavy chain of humanized antibody
atgggttggactcttgttttcttgttcctgttgagtgtgactgccggagtacactctcaggtgcaactccaacagagcggcgctgaggtggttcgaccaggcgcatccgtgaaggtgtcatgcaaagctagcgactacacctttaccgactatgagatgcattgggttaagcaggctcctggacaagggctggagtggataggcgctattcatcctggcaggggtggaaccgcatataaccagaagttcaaaggcagagtgacgatgacagccgataccagcatcagcacagcctatatggagctgtccagacttcgatccgacgataccgccgtctattactgcactagttatcacggcggttattggggtcagggtacaactctgacagtaagttctgcctctacgaaaggtccctccgtctttcccctcgcaccttcttccaagagcacaagtggaggaacagcagccctggggtgtttggtgaaggactacttcccagaacctgtgaccgtgagttggaattctggtgccctgacatccggggtccatacctttcccgcagtgcttcagtccagtggactctactctctgtctagcgttgtcaccgtgccctcatctagcctgggcacacagacctacatctgtaacgtgaatcacaaaccctccaacactaaagtcgacaagaaagtggaacctaagagctgcgataagacccatacatgcccaccatgtcctgctcctgaacttcttggcgggccatcagtgtttctgttccctccaaaacccaaggacaccctcatgattagcaggacaccagaagtcacctgtgtggtggtcgacgtatctcacgaggatccagaggtgaaatttaactggtatgtagacggcgttgaggtgcataatgccaagactaaaccccgggaagaacagtacaactccacctatcgcgtagtctcagttctgactgtgctgcaccaggattggttgaacgggaaggagtacaagtgtaaagtcagtaacaaagctctgccagctcccatcgaaaagaccatctcaaaggccaaggggcagcctcgtgaaccccaggtctacactctcccacccagccgggatgaactgacgaagaatcaggtatcactgacatgcctggtcaaaggcttttatcccagtgacattgccgtggagtgggagtccaatggacaacctgagaacaactacaagacaactcctcccgttctggatagcgatgggtccttcttcctgtacagcaagctcactgttgacaaatcacgctggcagcagggaaatgtgttttcctgctctgtgatgcatgaggctctgcacaatcactacacccagaagtccctgtccttgtctcccggcaag

SEQ ID NO: 69 - protein, 463 aa, Artificial Sequence
  Heavy chain of humanized antibody
MGWTLVFLFLLSVTAGVHSQVQLQQSGAEVVRPGASVKVSCKASDYTFTDYEMHWVKQAPGQGLEWIGAIHPGRGGTAYNQKFKGRVTMTADTSISTAYMELSRLRSDDTAVYYCTSYHGGYWGQGTTLTVSSASTKGPSVFPLAPSSKSTSGGTAALGCLVKDYFPEPVTVSWNSGALTSGVHTFPAVLQSSGLYSLSSVVTVPSSSLGTQTYICNVNHKPSNTKVDKKVEPKSCDKTHTCPPCPAPELLGGPSVFLFPPKPKDTLMISRTPEVTCVVVDVSHEDPEVKFNWYVDGVEVHNAKTKPREEQYNSTYRVVSVLTVLHQDWLNGKEYKCKVSNKALPAPIEKTISKAKGQPREPQVYTLPPSRDELTKNQVSLTCLVKGFYPSDIAVEWESNGQPENNYKTTPPVLDSDGSFFLYSKLTVDKSRWQQGNVFSCSVMHEALHNHYTQKSLSLSPGK

SEQ ID NO: 70 - DNA, 1389 bp, Artificial Sequence
  Heavy chain of humanized antibody
atgggatggacactggtgtttctgttccttctcagtgtgacagctggggtccattcccaagtgcaactgcagcaatcaggcgctgaagttaagcggccaggtgctagcgtaaaagtctcttgcaaggcatccgactacacatttaccgactatgagatgcactgggtgcgtcagacacctgggcatggtctggagtggatgggagccattcacccaggaagaggaggcactgcctacaatcagaagttcaaaggaagggttaccatgaccgctgataagtctacatctaccgtctacatggagctgagttccctgacttccgaggatactgccgtgtactactgcacatcctaccacggcggatattggggccaggggaccaccttgacagtctcctccgcttctaccaagggcccatctgtgtttcctctggccccatccagcaaaagtacttcaggtggcaccgctgcattgggctgtctggtgaaggactattttcctgaacccgtgacggtttcctggaattccggtgcactgacatccggggtgcatacatttcccgctgttctgcagagttctgggctttacagcctgagctctgtggtcactgtacccagtagctcattggggacccagacctatatctgcaatgtcaatcacaaaccctccaatacaaaagtcgacaagaaggtggaaccaaagtcatgtgacaagacgcatacttgcccaccctgtcccgcacccgaactgcttggtggcccttccgtattcctctttccacccaagcctaaagacaccttgatgatctctaggaccccagaagtgacttgcgtcgtagtggatgtatcccacgaagatccagaggtgaagttcaactggtatgtggacggtgttgaggtccacaacgccaaaactaagcctcgcgaagagcagtataacagcacctatcgggtcgtttctgtgctcacagttctgcatcaggactggctgaatggcaaggagtacaagtgtaaagtgagcaacaaagcccttcctgcccctattgagaaaacaatcagcaaggcaaagggccaacccagagagccccaggtctacactctgcctccctcacgcgacgagctcactaagaaccaggtttcactgacttgtctcgtgaagggtttctatcccagcgatatagccgtggaatgggagtctaatggacagcccgaaaacaactacaagaccaccccacctgtattggatagcgatggaagtttcttcctgtattctaagctgacggtggataaaagccgatggcagcaggggaacgtgtttagctgctctgtgatgcatgaggccctccacaaccactacacccagaaatcacttagtctgagtcctggcaaa

SEQ ID NO: 71 - protein, 463 aa, Artificial Sequence
  Heavy chain of humanized antibody
MGWTLVFLFLLSVTAGVHSQVQLQQSGAEVKRPGASVKVSCKASDYTFTDYEMHWVRQTPGHGLEWMGAIHPGRGGTAYNQKFKGRVTMTADKSTSTVYMELSSLTSEDTAVYYCTSYHGGYWGQGTTLTVSSASTKGPSVFPLAPSSKSTSGGTAALGCLVKDYFPEPVTVSWNSGALTSGVHTFPAVLQSSGLYSLSSVVTVPSSSLGTQTYICNVNHKPSNTKVDKKVEPKSCDKTHTCPPCPAPELLGGPSVFLFPPKPKDTLMISRTPEVTCVVVDVSHEDPEVKFNWYVDGVEVHNAKTKPREEQYNSTYRVVSVLTVLHQDWLNGKEYKCKVSNKALPAPIEKTISKAKGQPREPQVYTLPPSRDELTKNQVSLTCLVKGFYPSDIAVEWESNGQPENNYKTTPPVLDSDGSFFLYSKLTVDKSRWQQGNVFSCSVMHEALHNHYTQKSLSLSPGK

SEQ ID NO: 72 - DNA, 717 bp, Artificial Sequence
  Light chain of chimeric antibody
atggttagctccgctcagtttctgggacttctgctgttgtgctttcaagggactcggtgtgatgttgtcatgacgcaaacacccctgtcactgcctgtgtcactgggagatcaggcctccattagttgcagaagttctcagtccttggtgcactcaaatgagaacacctaccttctgtggtatctgcagaaaccaggccagtctcccaagctcctgatctacaaggtgtctaatcgcttcagtggcgttcctgacaggtttagtgggtccggttcagggaccgatttcaccctcaagataagccgagtagaggcagaggatcttggcgtttacttctgcagtcagacaactcatgtgccatggacttttggcggtggcaccaaactggagattaagcgtacagtggcagctccatctgtgttcatctttcctcccagcgatgagcagctgaaatccgggacagcttccgtcgtgtgtttgctcaacaacttctatcccagggaagccaaggtacagtggaaggtcgacaatgccctccagtcaggaaactcccaagagagcgtgaccgaacaggactccaaagactccacctatagcttgtctagcactctcactctgtctaaagccgactacgagaagcacaaggtgtatgcctgtgaagtcacccatcagggactgtctagccctgtcacaaagagcttcaatcggggtgaatgc

SEQ ID NO: 73 - protein, 239 aa, Artificial Sequence
  Light chain of chimeric antibody
MVSSAQFLGLLLLCFQGTRCDVVMTQTPLSLPVSLGDQASISCRSSQSLVHSNENTYLLWYLQKPGQSPKLLIYKVSNRFSGVPDRFSGSGSGTDFTLKISRVEAEDLGVYFCSQTTHVPWTFGGGTKLEIKRTVAAPSVFIFPPSDEQLKSGTASVVCLLNNFYPREAKVQWKVDNALQSGNSQESVTEQDSKDSTYSLSSTLTLSKADYEKHKVYACEVTHQGLSSPVTKSFNRGEC

SEQ ID NO: 74 - DNA, 717 bp, Artificial Sequence
  Light chain of humanized antibody
atggtgagctctgcccagtttctgggcctgttgctcctgtgctttcagggtacacgatgtgacatcgtgatgacgcagactcctctgtctagtcccgtgactcttggccagcctgcatccattagttgcaggagttctcagagcctggtccatagcaacgagaacacctatctgctctggtatctgcaaagacccggtcaaccacccaaactgctcatctacaaggtgtccaatcgcttttctggggttccagacaggttctcaggatccggtgcaggaaccgatttcacgctgaagattagccgtgtagaagccgaggatgtaggcgtgtacttctgctcccagactacccatgttccctggacatttgggcagggaaccaagttggagataaaacggactgtcgcagctccttccgtgttcatctttcctccctctgatgagcagctgaaatccgggacagcttccgtggtttgcttgctcaacaacttctatccaagagaagccaaagtccagtggaaggtcgacaatgctctgcagtcaggcaattcacaggagtctgtgacagagcaagactccaaggatagtacctactcccttagctctacccttaccctgagtaaagccgactacgaaaagcacaaggtctatgcctgtgaagtgacacaccaaggcctgtcaagcccagttactaagagcttcaatcggggagagtgt

SEQ ID NO: 75 - protein, 239 aa, Artificial Sequence
  Light chain of humanized antibody
MVSSAQFLGLLLLCFQGTRCDIVMTQTPLSSPVTLGQPASISCRSSQSLVHSNENTYLLWYLQRPGQPPKLLIYKVSNRFSGVPDRFSGSGAGTDFTLKISRVEAEDVGVYFCSQTTHVPWTFGQGTKLEIKRTVAAPSVFIFPPSDEQLKSGTASVVCLLNNFYPREAKVQWKVDNALQSGNSQESVTEQDSKDSTYSLSSTLTLSKADYEKHKVYACEVTHQGLSSPVTKSFNRGEC

SEQ ID NO: 76 - DNA, 717 bp, Artificial Sequence
  Light chain of humanized antibody
atggtcagctcagcccagtttctgggactcctcttgctgtgctttcagggcactcgttgcgacatagtcatgacacaatcaccactgtccctttctgtgacacctggacagccagcttccatttcctgccggtctagtcagtctctggtccatagcaacgagaacacctatcttctgtggtatctccagaagcctgggcaatctccccagttgctcatctacaaggtgtccaataggttctcaggtgttcccgatcgctttagcggatctgggtcaggtaccgacttcaccctgaagatcagtagggtggaagccgaggatgtgggcgtgtacttctgttcccagacaacacacgtaccctggacgtttggacaagggaccaaagtggagattaagcggaccgttgcagctcctagtgtgtttatcttccctccatctgatgagcagctgaagagcggcactgctagtgtagtctgtctgctgaacaacttctatcccagagaagccaaagtccagtggaaggtggacaatgccctgcaatccggcaatagccaggagagcgttaccgaacaggactctaaggatagcacatactccctttcctccactctgactctgtctaaagccgactacgagaaacacaaagtgtatgcatgtgaggtgactcatcagggtttgagtagccccgttaccaagtcattcaatcgaggcgaatgc

SEQ ID NO: 77 - protein, 239 aa, Artificial Sequence
  Light chain of humanized antibody
MVSSAQFLGLLLLCFQGTRCDIVMTQSPLSLSVTPGQPASISCRSSQSLVHSNENTYLLWYLQKPGQSPQLLIYKVSNRFSGVPDRFSGSGSGTDFTLKISRVEAEDVGVYFCSQTTHVPWTFGQGTKVEIKRTVAAPSVFIFPPSDEQLKSGTASVVCLLNNFYPREAKVQWKVDNALQSGNSQESVTEQDSKDSTYSLSSTLTLSKADYEKHKVYACEVTHQGLSSPVTKSFNRGEC

SEQ ID NO: 78 - DNA, 717 bp, Artificial Sequence
  Light chain of humanized antibody
atggtcagttctgcccaattccttgggctgcttctgctctgctttcagggcacaagatgcgacattcagatgacccagtcaccttcctctctgtccgctagtgtgggagatagggtcaccattacatgtcgctcatcccagtcactggttcacagcaatgagaacacctacctgttgtggtatctgcagaaacccggtcaagcacccaaactgctgatctacaaggtgtctaatcggttctcaggagtaccatcccggtttagcggaagtgggtctggcactgactttaccctgaccatctcttcactgcaacctgaggatttcgccacctacttttgctcccagacgactcatgtgccttggacatttggtggcggtaccaagctcgagataaagcgtaccgttgctgctccctccgtgttcatctttccaccttccgatgaacagctgaagtccggaactgcatctgtcgtgtgtttgctgaacaacttctatcccagggaagccaaagtgcagtggaaggttgacaacgcactgcagtctggcaattcccaggagagtgtaacagagcaggatagcaaagacagcacgtactctttgtccagcacactcactctcagcaaagccgactatgagaagcacaaggtgtatgcctgtgaagtcacacatcaagggcttagcagtccagtgactaagagcttcaatcgaggcgaatgc

SEQ ID NO: 79 - protein, 239 aa, Artificial Sequence
  Light chain of humanized antibody
MVSSAQFLGLLLLCFQGTRCDIQMTQSPSSLSASVGDRVTITCRSSQSLVHSNENTYLLWYLQKPGQAPKLLIYKVSNRFSGVPSRFSGSGSGTDFTLTISSLQPEDFATYFCSQTTHVPWTFGGGTKLEIKRTVAAPSVFIFPPSDEQLKSGTASVVCLLNNFYPREAKVQWKVDNALQSGNSQESVTEQDSKDSTYSLSSTLTLSKADYEKHKVYACEVTHQGLSSPVTKSFNRGEC